European Patent Application EP 4 722 391 A1, published April 8, 2026. Title: Primer set for detecting Carbapenemase-producing Enterobacteriaceae, detection method, and detection kit. Applicant: 慶應義塾. The sequence listing filed with the application follows.

SEQUENCE LISTING (33 sequences)

SEQ ID NO: 1 - DNA, 17 bp, synthetic construct
  source 1..17: mol_type = other DNA
tcgataccgcctggacc

SEQ ID NO: 2 - DNA, 19 bp, synthetic construct
  source 1..19: mol_type = other DNA
tcgacaacgcattggcata

SEQ ID NO: 3 - DNA, 37 bp, synthetic construct
  source 1..37: mol_type = other DNA
gcgcgaccggcaggttgatgatgaccagaccgcccag

SEQ ID NO: 4 - DNA, 35 bp, synthetic construct
  source 1..35: mol_type = other DNA
cggtggtgactcacgcgcaagtcgcaatccccgcc

SEQ ID NO: 5 - DNA, 18 bp, synthetic construct
  source 1..18: mol_type = other DNA
aatagcttgatcgccctc

SEQ ID NO: 6 - DNA, 21 bp, synthetic construct
  source 1..21: mol_type = other DNA
ccataatcgaaagcatgtagc

SEQ ID NO: 7 - DNA, 40 bp, synthetic construct
  source 1..40: mol_type = other DNA
gattccaagtggcgatatcgcggcgtggttaaggatgaac

SEQ ID NO: 8 - DNA, 43 bp, synthetic construct
  source 1..43: mol_type = other DNA
taatcaccgcgatgaaatattcagtcttgctcatacgtgcctc

SEQ ID NO: 9 - DNA, 20 bp, synthetic construct
  source 1..20: mol_type = other DNA
gcgtctgtccatcccactta

SEQ ID NO: 10 - DNA, 20 bp, synthetic construct
  source 1..20: mol_type = other DNA
gaatttgcccgccaaattgg

SEQ ID NO: 11 - DNA, 19 bp, synthetic construct
  source 1..19: mol_type = other DNA
gcgttgttcctaaacatgg

SEQ ID NO: 12 - DNA, 22 bp, synthetic construct
  source 1..22: mol_type = other DNA
ttgttaattcagatgcatacgt

SEQ ID NO: 13 - DNA, 46 bp, synthetic construct
  source 1..46: mol_type = other DNA
tccacaaaccaagtgactaactttttggttcttgtaaatgctgagg

SEQ ID NO: 14 - DNA, 45 bp, synthetic construct
  source 1..45: mol_type = other DNA
cgtggctataaaataaaaggcagcagatcgagaattaagccactc

SEQ ID NO: 15 - DNA, 25 bp, synthetic construct
  source 1..25: mol_type = other DNA
agtatctttagccgtaaatggagtg

SEQ ID NO: 16 - DNA, 19 bp, synthetic construct
  source 1..19: mol_type = other DNA
cgacagcacgggcggaata

SEQ ID NO: 17 - DNA, 17 bp, synthetic construct
  source 1..17: mol_type = other DNA
actccgccatcccaagc

SEQ ID NO: 18 - DNA, 17 bp, synthetic construct
  source 1..17: mol_type = other DNA
tccgactgcccagtctg

SEQ ID NO: 19 - DNA, 39 bp, synthetic construct
  source 1..39: mol_type = other DNA
tgcagagcccagtgtcagttttgatgcgcgcgatacctc

SEQ ID NO: 20 - DNA, 36 bp, synthetic construct
  source 1..36: mol_type = other DNA
gcagcggcagcagtttgttgcggatgcggtggttgc

SEQ ID NO: 21 - DNA, 20 bp, synthetic construct
  source 1..20: mol_type = other DNA
gtaagctttccgtcacggcg

SEQ ID NO: 22 - DNA, 22 bp, synthetic construct
  source 1..22: mol_type = other DNA
ttggctaaagggaaacacgacc

SEQ ID NO: 23 - DNA, 18 bp, synthetic construct
  source 1..18: mol_type = other DNA
aattccggtcggagaggt

SEQ ID NO: 24 - DNA, 18 bp, synthetic construct
  source 1..18: mol_type = other DNA
aaagtgcgtggagactgc

SEQ ID NO: 25 - DNA, 38 bp, synthetic construct
  source 1..38: mol_type = other DNA
cattggacgggtagaccgcgccagattgccgatggtgt

SEQ ID NO: 26 - DNA, 41 bp, synthetic construct
  source 1..41: mol_type = other DNA
tgattgatacagcgtggggtgcacgggaagtccaatttgct

SEQ ID NO: 27 - DNA, 20 bp, synthetic construct
  source 1..20: mol_type = other DNA
ccatcaaacgactgcgttgc

SEQ ID NO: 28 - DNA, 18 bp, synthetic construct
  source 1..18: mol_type = other DNA
tggtcgcatatcgcaacg

SEQ ID NO: 29 - DNA, 18 bp, synthetic construct
  source 1..18: mol_type = other DNA
gcccgaaggacatcaacg

SEQ ID NO: 30 - DNA, 41 bp, synthetic construct
  source 1..41: mol_type = other DNA
gcaccccacgctgtatcaatcaggtctacccgtccaatggt

SEQ ID NO: 31 - DNA, 39 bp, synthetic construct
  source 1..39: mol_type = other DNA
aacacagcggcacttctcgctgaaagtgcgtggagactg

SEQ ID NO: 32 - DNA, 24 bp, synthetic construct
  source 1..24: mol_type = other DNA
gcaactcatcaccatcacggacaa

SEQ ID NO: 33 - DNA, 22 bp, synthetic construct
  source 1..22: mol_type = other DNA
gcaaattggacttcccgtaacg